European Patent Specification EP 3 912 955 B1, published January 1, 2025. Title: GRAPHENE-INDUCED ENERGY TRANSFER FOR THE QUANTIFICATION OF THE STRUCTURE AND DYNAMICS OF BIOMOLECULES. Applicant: Universität Osnabrück. Application not yet assigned. The sequence listing filed with the application follows.

SEQUENCE LISTING (8 sequences)

SEQ ID NO: 1 - DNA, 20 bp, Artificial Sequence
  DNA strand
  3'-TEG-Cholesterol
gatgaatggtgggtgagagg

SEQ ID NO: 2 - DNA, 25 bp, Artificial Sequence
  DNA strand
  3'-Cholesterol
gatgaatggtgggtgagaggtgagg

SEQ ID NO: 3 - DNA, 35 bp, Artificial Sequence
  DNA strand
  3'-Cholesterol
gatgaatggtgggtgagaggtgaggagtaagagga

SEQ ID NO: 4 - DNA, 50 bp, Artificial Sequence
  DNA strand
  3'-Cholesterol
gatgaatggtgggtgagaggtgaggagtaagaggatgtgttagagggatg

SEQ ID NO: 5 - DNA, 20 bp, Artificial Sequence
  DNA strand
  3'-FAM
cctctcacccaccattcatc

SEQ ID NO: 6 - DNA, 20 bp, Artificial Sequence
  DNA strand
  5'-FAM
cctctcacccaccattcatc

SEQ ID NO: 7 - DNA, 15 bp, Artificial Sequence
  DNA strand
tcctcttactcctca

SEQ ID NO: 8 - DNA, 30 bp, Artificial Sequence
  DNA strand
catccctctaacacatcctcttactcctca